European Patent Application EP 4 331 619 A1, published March 6, 2024. Title: Therapeutic agent for myotonic dystrophy type 1. Applicant: EditForce, Inc. Osaka University. The sequence listing filed with the application follows.

SEQUENCE LISTING (29 sequences)

SEQ ID NO: 1 - protein, 35 aa, Artificial Sequence
  Artificial polypeptide
VTYNTLIDGLCKSGKIEEALKLFKEMEEKGITPSV

SEQ ID NO: 2 - protein, 35 aa, Artificial Sequence
  Artificial polypeptide
VTYNTNIDQLCKSGKIEEALKLFKEMEEKGITPSV

SEQ ID NO: 3 - protein, 35 aa, Artificial Sequence
  Artificial polypeptide
VTYNTNIDQLCKSGRIEEALKLFKEMEEKGITPSV

SEQ ID NO: 4 - protein, 35 aa, Artificial Sequence
  Artificial polypeptide
VTYNTLIDGLCKSGRIEEALKLFKEMEEKGITPSV

SEQ ID NO: 5 - protein, 35 aa, Artificial Sequence
  Artificial polypeptide
VTYNTLIDGLCKAGRLDEAEELLEEMEEKGIKPDV

SEQ ID NO: 6 - protein, 35 aa, Artificial Sequence
  Artificial polypeptide
VTYNTLIDGLCKAGKLDEAEELLEEMEEKGIKPDV

SEQ ID NO: 7 - protein, 35 aa, Artificial Sequence
  Artificial polypeptide
VTYTTLIDGLCKAGKVDEALELFDEMKERGIKPDV

SEQ ID NO: 8 - protein, 35 aa, Artificial Sequence
  Artificial polypeptide
VTYTTLIDGLCKAGKVDEALELFDEMKERGIKPDE

SEQ ID NO: 9 - protein, 35 aa, Artificial Sequence
  Artificial polypeptide
VTYTTLIDGLCKAGRVDEALELFDEMKERGIKPDV

SEQ ID NO: 10 - protein, 35 aa, Artificial Sequence
  Artificial polypeptide
VTYTTLIDGLCKAGRVDEALELFDEMKERGIKPDE

SEQ ID NO: 11 - protein, 869 aa, Artificial Sequence
  Artificial polypeptide
MAGVFTLEDFVGDWRQTAGYNLDQVLEQGGVSSLFQNLGVSVTPIQRIVLSGENGLKIDIHVIIPYEGLSGDQMGQIEKIFKVVYPVDDHHFKVILHYGTLVIDGVTPNMIDYFGRPYEGIAVFDGKKITVTGTLWNGNKIIDERLINPDGSLLFRVTINGVTGWRLCERILAGGGGSLVPRGSGGGGSSRLHMGNSVVTYNTLIDGLCKSGKIEEALKLFKEMEEKGITPSVVTYNTLIDGLCKAGRLDEAEELLEEMEEKGIKPDVVTYTTLIDGLCKAGKVDEALELFDEMKERGIKPDVVTYNTLIDGLCKSGKIEEALKLFKEMEEKGITPSVVTYNTLIDGLCKAGRLDEAEELLEEMEEKGIKPDVVTYTTLIDGLCKAGKVDEALELFDEMKERGIKPDVVTYNTLIDGLCKSGKIEEALKLFKEMEEKGITPSVVTYNTLIDGLCKAGRLDEAEELLEEMEEKGIKPDVVTYTTLIDGLCKAGKVDEALELFDEMKERGIKPDVVTYNTLIDGLCKSGKIEEALKLFKEMEEKGITPSVVTYNTLIDGLCKAGRLDEAEELLEEMEEKGIKPDVVTYTTLIDGLCKAGKVDEALELFDEMKERGIKPDVVTYNTLIDGLCKSGKIEEALKLFKEMEEKGITPSVVTYNTLIDGLCKAGRLDEAEELLEEMEEKGIKPDVVTYTTLIDGLCKAGKVDEALELFDEMKERGIKPDVVTYNTLIDGLCKSGKIEEALKLFKEMEEKGITPSVVTYNTLIDGLCKAGRLDEAEELLEEMEEKGIKPDVVTYTTLIDGLCKAGKVDEALELFDEMKERGIKPDELTYNTLISGLGKAGRARDPPVLSSGSGGSGGGGHHHHHHGR

SEQ ID NO: 12 - protein, 869 aa, Artificial Sequence
  Artificial polypeptide
MAGVFTLEDFVGDWRQTAGYNLDQVLEQGGVSSLFQNLGVSVTPIQRIVLSGENGLKIDIHVIIPYEGLSGDQMGQIEKIFKVVYPVDDHHFKVILHYGTLVIDGVTPNMIDYFGRPYEGIAVFDGKKITVTGTLWNGNKIIDERLINPDGSLLFRVTINGVTGWRLCERILAGGGGSLVPRGSGGGGSSRLHMGNSVVTYNTNIDQLCKSGKIEEALKLFKEMEEKGITPSVVTYNTLIDGLCKAGRLDEAEELLEEMEEKGIKPDVVTYTTLIDGLCKAGKVDEALELFDEMKERGIKPDVVTYNTLIDGLCKSGKIEEALKLFKEMEEKGITPSVVTYNTLIDGLCKAGRLDEAEELLEEMEEKGIKPDVVTYTTLIDGLCKAGKVDEALELFDEMKERGIKPDVVTYNTLIDGLCKSGKIEEALKLFKEMEEKGITPSVVTYNTLIDGLCKAGRLDEAEELLEEMEEKGIKPDVVTYTTLIDGLCKAGKVDEALELFDEMKERGIKPDVVTYNTLIDGLCKSGKIEEALKLFKEMEEKGITPSVVTYNTLIDGLCKAGRLDEAEELLEEMEEKGIKPDVVTYTTLIDGLCKAGKVDEALELFDEMKERGIKPDVVTYNTLIDGLCKSGKIEEALKLFKEMEEKGITPSVVTYNTLIDGLCKAGRLDEAEELLEEMEEKGIKPDVVTYTTLIDGLCKAGKVDEALELFDEMKERGIKPDVVTYNTLIDGLCKSGKIEEALKLFKEMEEKGITPSVVTYNTLIDGLCKAGRLDEAEELLEEMEEKGIKPDVVTYTTLIDGLCKAGKVDEALELFDEMKERGIKPDELTYNTLISGLGKAGRARDPPVLSSGSGGSGGGGHHHHHHGR

SEQ ID NO: 13 - protein, 869 aa, Artificial Sequence
  Artificial polypeptide
MAGVFTLEDFVGDWRQTAGYNLDQVLEQGGVSSLFQNLGVSVTPIQRIVLSGENGLKIDIHVIIPYEGLSGDQMGQIEKIFKVVYPVDDHHFKVILHYGTLVIDGVTPNMIDYFGRPYEGIAVFDGKKITVTGTLWNGNKIIDERLINPDGSLLFRVTINGVTGWRLCERILAGGGGSLVPRGSGGGGSSRLHMGNSVVTYNTNIDQLCKSGKIEEALKLFKEMEEKGITPSVVTYNTLIDGLCKAGKLDEAEELLEEMEEKGIKPDVVTYTTLIDGLCKAGKVDEALELFDEMKERGIKPDVVTYNTLIDGLCKSGKIEEALKLFKEMEEKGITPSVVTYNTLIDGLCKAGKLDEAEELLEEMEEKGIKPDVVTYTTLIDGLCKAGKVDEALELFDEMKERGIKPDVVTYNTLIDGLCKSGKIEEALKLFKEMEEKGITPSVVTYNTLIDGLCKAGKLDEAEELLEEMEEKGIKPDVVTYTTLIDGLCKAGKVDEALELFDEMKERGIKPDVVTYNTLIDGLCKSGKIEEALKLFKEMEEKGITPSVVTYNTLIDGLCKAGKLDEAEELLEEMEEKGIKPDVVTYTTLIDGLCKAGKVDEALELFDEMKERGIKPDVVTYNTLIDGLCKSGKIEEALKLFKEMEEKGITPSVVTYNTLIDGLCKAGKLDEAEELLEEMEEKGIKPDVVTYTTLIDGLCKAGKVDEALELFDEMKERGIKPDVVTYNTLIDGLCKSGKIEEALKLFKEMEEKGITPSVVTYNTLIDGLCKAGKLDEAEELLEEMEEKGIKPDVVTYTTLIDGLCKAGKVDEALELFDEMKERGIKPDELTYNTLISGLGKAGRARDPPVLSSGSGGSGGGGHHHHHHGR

SEQ ID NO: 14 - protein, 869 aa, Artificial Sequence
  Artificial polypeptide
MAGVFTLEDFVGDWRQTAGYNLDQVLEQGGVSSLFQNLGVSVTPIQRIVLSGENGLKIDIHVIIPYEGLSGDQMGQIEKIFKVVYPVDDHHFKVILHYGTLVIDGVTPNMIDYFGRPYEGIAVFDGKKITVTGTLWNGNKIIDERLINPDGSLLFRVTINGVTGWRLCERILAGGGGSLVPRGSGGGGSSRLHMGNSVVTYNTNIDQLCKSGRIEEALKLFKEMEEKGITPSVVTYNTLIDGLCKAGRLDEAEELLEEMEEKGIKPDVVTYTTLIDGLCKAGRVDEALELFDEMKERGIKPDVVTYNTLIDGLCKSGRIEEALKLFKEMEEKGITPSVVTYNTLIDGLCKAGRLDEAEELLEEMEEKGIKPDVVTYTTLIDGLCKAGRVDEALELFDEMKERGIKPDVVTYNTLIDGLCKSGRIEEALKLFKEMEEKGITPSVVTYNTLIDGLCKAGRLDEAEELLEEMEEKGIKPDVVTYTTLIDGLCKAGRVDEALELFDEMKERGIKPDVVTYNTLIDGLCKSGRIEEALKLFKEMEEKGITPSVVTYNTLIDGLCKAGRLDEAEELLEEMEEKGIKPDVVTYTTLIDGLCKAGRVDEALELFDEMKERGIKPDVVTYNTLIDGLCKSGRIEEALKLFKEMEEKGITPSVVTYNTLIDGLCKAGRLDEAEELLEEMEEKGIKPDVVTYTTLIDGLCKAGRVDEALELFDEMKERGIKPDVVTYNTLIDGLCKSGRIEEALKLFKEMEEKGITPSVVTYNTLIDGLCKAGRLDEAEELLEEMEEKGIKPDVVTYTTLIDGLCKAGRVDEALELFDEMKERGIKPDELTYNTLISGLGKAGRARDPPVLSSGSGGSGGGGHHHHHHGR

SEQ ID NO: 15 - RNA, 30 nt, Artificial Sequence
  Artificial polynucleotide
gacacugcugcugcugcugcugcugaugca

SEQ ID NO: 16 - RNA, 30 nt, Artificial Sequence
  Artificial polynucleotide
gacaugccagcagcagcagcagcaggacug

SEQ ID NO: 17 - protein, 957 aa, Artificial Sequence
  Artificial polypeptide
MAGVSKGEELFTGVVPILVELDGDVNGHKFSVRGEGEGDATNGKLTLKFICTTGKLPVPWPTLVTTFGYGVACFSRYPDHMKQHDFFKSAMPEGYVQERTISFKDDGTYKTRAEVKFEGDTLVNRIELKGIDFKEDGNILGHKLEYNFNSHYVYITADKQKNCIKANFKIRHNVEDGSVQLADHYQQNTPIGDGPVLLPDNHYLSHQSKLSKDPNEKRDHMVLLEFVTAAGITHGMDELYKSRLHMGNSVVTYNTLIDGLCKSGKIEEALKLFKEMEEKGITPSVVTYNTLIDGLCKAGRLDEAEELLEEMEEKGIKPDVVTYTTLIDGLCKAGKVDEALELFDEMKERGIKPDVVTYNTLIDGLCKSGKIEEALKLFKEMEEKGITPSVVTYNTLIDGLCKAGRLDEAEELLEEMEEKGIKPDVVTYTTLIDGLCKAGKVDEALELFDEMKERGIKPDVVTYNTLIDGLCKSGKIEEALKLFKEMEEKGITPSVVTYNTLIDGLCKAGRLDEAEELLEEMEEKGIKPDVVTYTTLIDGLCKAGKVDEALELFDEMKERGIKPDVVTYNTLIDGLCKSGKIEEALKLFKEMEEKGITPSVVTYNTLIDGLCKAGRLDEAEELLEEMEEKGIKPDVVTYTTLIDGLCKAGKVDEALELFDEMKERGIKPDVVTYNTLIDGLCKSGKIEEALKLFKEMEEKGITPSVVTYNTLIDGLCKAGRLDEAEELLEEMEEKGIKPDVVTYTTLIDGLCKAGKVDEALELFDEMKERGIKPDVVTYNTLIDGLCKSGKIEEALKLFKEMEEKGITPSVVTYNTLIDGLCKAGRLDEAEELLEEMEEKGIKPDVVTYTTLIDGLCKAGKVDEALELFDEMKERGIKPDELTYNTLISGLGKAGRARDPPVLSSPKKKRKVEDPKKKRKVEDPKKKRKVGSDYKDHDGDYKDHDIDYKDDDDKMAGR

SEQ ID NO: 18 - protein, 957 aa, Artificial Sequence
  Artificial polypeptide
MAGVSKGEELFTGVVPILVELDGDVNGHKFSVRGEGEGDATNGKLTLKFICTTGKLPVPWPTLVTTFGYGVACFSRYPDHMKQHDFFKSAMPEGYVQERTISFKDDGTYKTRAEVKFEGDTLVNRIELKGIDFKEDGNILGHKLEYNFNSHYVYITADKQKNCIKANFKIRHNVEDGSVQLADHYQQNTPIGDGPVLLPDNHYLSHQSKLSKDPNEKRDHMVLLEFVTAAGITHGMDELYKSRLHMGNSVVTYNTNIDQLCKSGKIEEALKLFKEMEEKGITPSVVTYNTLIDGLCKAGRLDEAEELLEEMEEKGIKPDVVTYTTLIDGLCKAGKVDEALELFDEMKERGIKPDVVTYNTLIDGLCKSGKIEEALKLFKEMEEKGITPSVVTYNTLIDGLCKAGRLDEAEELLEEMEEKGIKPDVVTYTTLIDGLCKAGKVDEALELFDEMKERGIKPDVVTYNTLIDGLCKSGKIEEALKLFKEMEEKGITPSVVTYNTLIDGLCKAGRLDEAEELLEEMEEKGIKPDVVTYTTLIDGLCKAGKVDEALELFDEMKERGIKPDVVTYNTLIDGLCKSGKIEEALKLFKEMEEKGITPSVVTYNTLIDGLCKAGRLDEAEELLEEMEEKGIKPDVVTYTTLIDGLCKAGKVDEALELFDEMKERGIKPDVVTYNTLIDGLCKSGKIEEALKLFKEMEEKGITPSVVTYNTLIDGLCKAGRLDEAEELLEEMEEKGIKPDVVTYTTLIDGLCKAGKVDEALELFDEMKERGIKPDVVTYNTLIDGLCKSGKIEEALKLFKEMEEKGITPSVVTYNTLIDGLCKAGRLDEAEELLEEMEEKGIKPDVVTYTTLIDGLCKAGKVDEALELFDEMKERGIKPDELTYNTLISGLGKAGRARDPPVLSSPKKKRKVEDPKKKRKVEDPKKKRKVGSDYKDHDGDYKDHDIDYKDDDDKMAGR

SEQ ID NO: 19 - protein, 957 aa, Artificial Sequence
  Artificial polypeptide
MAGVSKGEELFTGVVPILVELDGDVNGHKFSVRGEGEGDATNGKLTLKFICTTGKLPVPWPTLVTTFGYGVACFSRYPDHMKQHDFFKSAMPEGYVQERTISFKDDGTYKTRAEVKFEGDTLVNRIELKGIDFKEDGNILGHKLEYNFNSHYVYITADKQKNCIKANFKIRHNVEDGSVQLADHYQQNTPIGDGPVLLPDNHYLSHQSKLSKDPNEKRDHMVLLEFVTAAGITHGMDELYKSRLHMGNSVVTYNTNIDQLCKSGKIEEALKLFKEMEEKGITPSVVTYNTLIDGLCKAGKLDEAEELLEEMEEKGIKPDVVTYTTLIDGLCKAGKVDEALELFDEMKERGIKPDVVTYNTLIDGLCKSGKIEEALKLFKEMEEKGITPSVVTYNTLIDGLCKAGKLDEAEELLEEMEEKGIKPDVVTYTTLIDGLCKAGKVDEALELFDEMKERGIKPDVVTYNTLIDGLCKSGKIEEALKLFKEMEEKGITPSVVTYNTLIDGLCKAGKLDEAEELLEEMEEKGIKPDVVTYTTLIDGLCKAGKVDEALELFDEMKERGIKPDVVTYNTLIDGLCKSGKIEEALKLFKEMEEKGITPSVVTYNTLIDGLCKAGKLDEAEELLEEMEEKGIKPDVVTYTTLIDGLCKAGKVDEALELFDEMKERGIKPDVVTYNTLIDGLCKSGKIEEALKLFKEMEEKGITPSVVTYNTLIDGLCKAGKLDEAEELLEEMEEKGIKPDVVTYTTLIDGLCKAGKVDEALELFDEMKERGIKPDVVTYNTLIDGLCKSGKIEEALKLFKEMEEKGITPSVVTYNTLIDGLCKAGKLDEAEELLEEMEEKGIKPDVVTYTTLIDGLCKAGKVDEALELFDEMKERGIKPDELTYNTLISGLGKAGRARDPPVLSSPKKKRKVEDPKKKRKVEDPKKKRKVGSDYKDHDGDYKDHDIDYKDDDDKMAGR

SEQ ID NO: 20 - protein, 957 aa, Artificial Sequence
  Artificial polypeptide
MAGVSKGEELFTGVVPILVELDGDVNGHKFSVRGEGEGDATNGKLTLKFICTTGKLPVPWPTLVTTFGYGVACFSRYPDHMKQHDFFKSAMPEGYVQERTISFKDDGTYKTRAEVKFEGDTLVNRIELKGIDFKEDGNILGHKLEYNFNSHYVYITADKQKNCIKANFKIRHNVEDGSVQLADHYQQNTPIGDGPVLLPDNHYLSHQSKLSKDPNEKRDHMVLLEFVTAAGITHGMDELYKSRLHMGNSVVTYNTNIDQLCKSGRIEEALKLFKEMEEKGITPSVVTYNTLIDGLCKAGRLDEAEELLEEMEEKGIKPDVVTYTTLIDGLCKAGRVDEALELFDEMKERGIKPDVVTYNTLIDGLCKSGRIEEALKLFKEMEEKGITPSVVTYNTLIDGLCKAGRLDEAEELLEEMEEKGIKPDVVTYTTLIDGLCKAGRVDEALELFDEMKERGIKPDVVTYNTLIDGLCKSGRIEEALKLFKEMEEKGITPSVVTYNTLIDGLCKAGRLDEAEELLEEMEEKGIKPDVVTYTTLIDGLCKAGRVDEALELFDEMKERGIKPDVVTYNTLIDGLCKSGRIEEALKLFKEMEEKGITPSVVTYNTLIDGLCKAGRLDEAEELLEEMEEKGIKPDVVTYTTLIDGLCKAGRVDEALELFDEMKERGIKPDVVTYNTLIDGLCKSGRIEEALKLFKEMEEKGITPSVVTYNTLIDGLCKAGRLDEAEELLEEMEEKGIKPDVVTYTTLIDGLCKAGRVDEALELFDEMKERGIKPDVVTYNTLIDGLCKSGRIEEALKLFKEMEEKGITPSVVTYNTLIDGLCKAGRLDEAEELLEEMEEKGIKPDVVTYTTLIDGLCKAGRVDEALELFDEMKERGIKPDELTYNTLISGLGKAGRARDPPVLSSPKKKRKVEDPKKKRKVEDPKKKRKVGSDYKDHDGDYKDHDIDYKDDDDKMAGR

SEQ ID NO: 21 - protein, 306 aa, Artificial Sequence
  Artificial polypeptide
MAGVSKGEELFTGVVPILVELDGDVNGHKFSVRGEGEGDATNGKLTLKFICTTGKLPVPWPTLVTTFGYGVACFSRYPDHMKQHDFFKSAMPEGYVQERTISFKDDGTYKTRAEVKFEGDTLVNRIELKGIDFKEDGNILGHKLEYNFNSHYVYITADKQKNCIKANFKIRHNVEDGSVQLADHYQQNTPIGDGPVLLPDNHYLSHQSKLSKDPNEKRDHMVLLEFVTAAGITHGMDELYKSRLHMGSGGLSSPKKKRKVEDPKKKRKVEDPKKKRKVGSDYKDHDGDYKDHDIDYKDDDDKMAGR

SEQ ID NO: 22 - DNA, 23 bp, Artificial Sequence
  Artificial polynucleotide
gctcatggtcctcaagatctcac

SEQ ID NO: 23 - DNA, 20 bp, Artificial Sequence
  Artificial polynucleotide
gggtcagtgcctcagctttg

SEQ ID NO: 24 - DNA, 24 bp, Artificial Sequence
  Artificial polynucleotide
tgaaggaatacctcacactcaagg

SEQ ID NO: 25 - DNA, 20 bp, Artificial Sequence
  Artificial polynucleotide
cacggaacacaaaggcactg

SEQ ID NO: 26 - DNA, 22 bp, Artificial Sequence
  Synthetic polynucleotides
gatgaggctttggaactgtttg

SEQ ID NO: 27 - DNA, 22 bp, Artificial Sequence
  Synthetic polynucleotides
tctctggctctgccggccttgc

SEQ ID NO: 28 - DNA, 20 bp, Artificial Sequence
  Synthetic polynucleotides
atcatccctgcctctactgg

SEQ ID NO: 29 - DNA, 20 bp, Artificial Sequence
  Synthetic polynucleotides
ctgcttcaccaccttcttga